European Patent Specification EP 3 765 511 B1, published July 24, 2024. Title: ANTI-CD25 ANTIBODY AGENTS. Applicant: TUSK THERAPEUTICS LTD CANCER RESEARCH TECHNOLOGY LIMITED. The sequence listing filed with the application follows.

SEQUENCE LISTING (7 sequences)

SEQ ID NO: 1 - protein, 123 aa, homo sapiens
EVQLLESGGGLVQPGGSLRLSCAASGFTFSSYGMSWVRQAPGKGLELVSTINGYGDTTYYPDSVKGRFTISRDNSKNTLYLQMNSLRAEDTAVYYCARDRDYGNSYYYALDYWGQGTLVTVSS

SEQ ID NO: 2 - protein, 123 aa, homo sapiens
EVQLLESGGGLVQPGGSLRLSCAASGFTFSSYGMSWVRQAPGKGLELVSTINGYGDTTYYPDSVKGRFTISRDNAKNTLYLQMNSLRAEDTAVYFCARDRDYGNSYYYALDYWGQGTLVTVSS

SEQ ID NO: 3 - protein, 106 aa, homo sapiens
EIVLTQSPGTLSLSPGERATLSCRASSSVSFMHWLQQKPGQAPRPLIYATSNLASGIPDRFSGSGSGTDYTLTISRLEPEDFAVYYCQQWSSNPPAFGQGTKLEIK

SEQ ID NO: 4 - protein, 106 aa, homo sapiens
QIVLTQSPGTLSLSPGERATLSCRASSSVSFMHWLQQKPGQSPRPLIYATSNLASGIPDRFSGSGSGTDYTLTISRLEPEDFAVYYCQQWSSNPPAFGQGTKLEIK

SEQ ID NO: 5 - protein, 272 aa, homo sapiens
MDSYLLMWGLLTFIMVPGCQAELCDDDPPEIPHATFKAMAYKEGTMLNCECKRGFRRIKSGSLYMLCTGNSSHSSWDNQCQCTSSATRNTTKQVTPQPEEQKERKTTEMQSPMQPVDQASLPGHCREPPPWENEATERIYHFVVGQMVYYQCVQGYRALHRGPAESVCKMTHGKTRWTQPQLICTGEMETSQFPGEEKPQASPEGRPESETSCLVTTTDFQIQTEMAATMETSIFTTEYQVAVAGCVFLLISVLLLSGLTWQRRQRKSRRTI

SEQ ID NO: 6 - protein, 14 aa, Homo sapiens
YQCVQGYRALHRGP

SEQ ID NO: 7 - protein, 15 aa, Homo sapiens
SVCKMTHGKTRWTQP